European Patent Specification EP 3 969 025 B1, published April 9, 2025. Title: Novel Compositions. Applicant: Intract Pharma Ltd. The sequence listing filed with the application follows.

SEQUENCE LISTING (1 sequence)

SEQ ID NO: 1 - protein, 58 aa, Homo sapiens
  Aprotinin
RPDFCLEPPYTGPCKARMIRYFYNAKAGLCQPFVYGGCRAKRNNFKSSEDCMRTCGGA